European Patent Specification EP 3 482 765 B1, published February 28, 2024. Title: LONG-ACTING GROWTH HORMONE AND METHODS OF PRODUCING SAME. Applicant: OPKO Biologics Ltd. The sequence listing filed with the application follows.

SEQUENCE LISTING (26 sequences)

SEQ ID NO: 1 - protein, 33 aa, Homo sapiens
DPRFQDSSSSKAPPPSLPSPSRLPGPSDTPILQ

SEQ ID NO: 2 - protein, 28 aa, Homo sapiens
SSSSKAPPPSLPSPSRLPGPSDTPILPQ

SEQ ID NO: 3 - protein, 26 aa, Homo sapiens
MATGSRTSLLLAFGLLCLPWLQEGSA

SEQ ID NO: 4 - protein, 12 aa, Homo sapiens
SSSSKAPPPSLP

SEQ ID NO: 5 - protein, 217 aa, Homo sapiens
MATGSRTSLLLAFGLLCLPWLQEGSAFPTIPLSRLFDNAMLRAHRLHQLAFDTYQEFEEAYIPKEQKYSFLQNPQTSLCFSESIPTPSNREETQQKSNLELLRISLLLIQSWLEPVQFLRSVFANSLVYGASDSNVYDLLKDLEEGIQTLMGRLEDGSPRTGQIFKQTYSKFDTNSHNDDALLKNYGLLYCFRKDMDKVETFLRIVQCRSVEGSCGF

SEQ ID NO: 6 - protein, 192 aa, Homo sapiens
MFPTIPLSRLFDNAMLRAHRLHQLAFDTYQEFEEAYIPKEQKYSFLQNPQTSLCFSESIPTPSNREETQQKSNLELLRISLLLIQSWLEPVQFLRSVFANSLVYGASDSNVYDLLKDLEEGIQTLMGRLEDGSPRTGQIFKQTYSKFDTNSHNDDALLKNYGLLYCFRKDMDKVETFLRIVQCRSVEGSCGF

SEQ ID NO: 7 - protein, 25 aa, Homo sapiens
MFPTIPLSRLFDNAMLRAHRLHQLA

SEQ ID NO: 8 - protein, 217 aa, Homo sapiens
MATGSRTSLLLAFGLLCLPWLQEGSAFPTIPLSRLFDNAMLRAHRLHQLAFDTYQEFEEAYIPKVQKYSFLQNPQTSLCFSESIPTPSNREETQQKSNLELLRISLLLIQSWLEPVQFLRSVFANSLVYGASDSNVYDLLKDLEEGIQTLMGRLEDGSPRTGQIFKQTYSKFDTNSHNDDALLKNYGLLYCFRKDMDKVETFLRIVQCRSVEGSCGF

SEQ ID NO: 9 - protein, 245 aa, Homo sapiens
MATGSRTSLLLAFGLLCLPWLQEGSAFPTIPLSRLFDNAMLRAHRLHQLAFDTYQEFEEAYIPKEQKYSFLQNPQTSLCFSESIPTPSNREETQQKSNLELLRISLLLIQSWLEPVQFLRSVFANSLVYGASDSNVYDLLKDLEEGIQTLMGRLEDGSPRTGQIFKQTYSKFDTNSHNDDALLKNYGLLYCFRKDMDKVETFLRIVQCRSVEGSCGFSSSSKAPPPSLPSPSRLPGPSDTPILPQ

SEQ ID NO: 10 - protein, 273 aa, Homo sapiens
MATGSRTSLLLAFGLLCLPWLQEGSAFPTIPLSRLFDNAMLRAHRLHQLAFDTYQEFEEAYIPKEQKYSFLQNPQTSLCFSESIPTPSNREETQQKSNLELLRISLLLIQSWLEPVQFLRSVFANSLVYGASDSNVYDLLKDLEEGIQTLMGRLEDGSPRTGQIFKQTYSKFDTNSHNDDALLKNYGLLYCFRKDMDKVETFLRIVQCRSVEGSCGFSSSSKAPPPSLPSPSRLPGPSDTPILPQSSSSKAPPPSLPSPSRLPGPSDTPILPQ

SEQ ID NO: 11 - protein, 301 aa, Homo sapiens
MATGSRTSLLLAFGLLCLPWLQEGSASSSSKAPPPSLPSPSRLPGPSDTPILPQFPTIPLSRLFDNAMLRAHRLHQLAFDTYQEFEEAYIPKEQKYSFLQNPQTSLCFSESIPTPSNREETQQKSNLELLRISLLLIQSWLEPVQFLRSVFANSLVYGASDSNVYDLLKDLEEGIQTLMGRLEDGSPRTGQIFKQTYSKFDTNSHNDDALLKNYGLLYCFRKDMDKVETFLRIVQCRSVEGSCGFSSSSKAPPPSLPSPSRLPGPSDTPILPQSSSSKAPPPSLPSPSRLPGPSDTPILPQ

SEQ ID NO: 12 - protein, 285 aa, Homo sapiens
MATGSRTSLLLAFGLLCLPWLQEGSASSSSKAPPPSLPFPTIPLSRLFDNAMLRAHRLHQLAFDTYQEFEEAYIPKEQKYSFLQNPQTSLCFSESIPTPSNREETQQKSNLELLRISLLLIQSWLEPVQFLRSVFANSLVYGASDSNVYDLLKDLEEGIQTLMGRLEDGSPRTGQIFKQTYSKFDTNSHNDDALLKNYGLLYCFRKDMDKVETFLRIVQCRSVEGSCGFSSSSKAPPPSLPSPSRLPGPSDTPILPQSSSSKAPPPSLPSPSRLPGPSDTPILPQ

SEQ ID NO: 13 - protein, 273 aa, Homo sapiens
MATGSRTSLLLAFGLLCLPWLQEGSASSSSKAPPPSLPSPSRLPGPSDTPILPQFPTIPLSRLFDNAMLRAHRLHQLAFDTYQEFEEAYIPKEQKYSFLQNPQTSLCFSESIPTPSNREETQQKSNLELLRISLLLIQSWLEPVQFLRSVFANSLVYGASDSNVYDLLKDLEEGIQTLMGRLEDGSPRTGQIFKQTYSKFDTNSHNDDALLKNYGLLYCFRKDMDKVETFLRIVQCRSVEGSCGFSSSSKAPPPSLPSPSRLPGPSDTPILPQ

SEQ ID NO: 14 - protein, 245 aa, Homo sapiens
MATGSRTSLLLAFGLLCLPWLQEGSASSSSKAPPPSLPSPSRLPGPSDTPILPQFPTIPLSRLFDNAMLRAHRLHQLAFDTYQEFEEAYIPKEQKYSFLQNPQTSLCFSESIPTPSNREETQQKSNLELLRISLLLIQSWLEPVQFLRSVFANSLVYGASDSNVYDLLKDLEEGIQTLMGRLEDGSPRTGQIFKQTYSKFDTNSHNDDALLKNYGLLYCFRKDMDKVETFLRIVQCRSVEGSCGF

SEQ ID NO: 15 - DNA, 853 bp, Homo sapiens
tctagaggacatggccaccggcagcaggaccagcctgctgctggccttcggcctgctgtgcctgccatggctgcaggagggcagcgccagctcttcttctaaggctccacccccatctctgcccagccccagcagactgccgggccccagcgacacacccattctgccccagttccccaccatccccctgagcaggctgttcgacaacgccatgctgagggctcacaggctgcaccagctggcctttgacacctaccaggagttcgaggaagcctacatccccaaggagcagaagtacagcttcctgcagaacccccagacctccctgtgcttcagcgagagcatccccacccccagcaacagagaggagacccagcagaagagcaacctggagctgctgaggatctccctgctgctgatccagagctggctggagcccgtgcagttcctgagaagcgtgttcgccaacagcctggtgtacggcgccagcgacagcaacgtgtacgacctgctgaaggacctggaggagggcatccagaccctgatgggccggctggaggacggcagccccaggaccggccagatcttcaagcagacctacagcaagttcgacaccaacagccacaacgacgacgccctgctgaagaactacgggctgctgtactgcttcagaaaggacatggacaaggtggagaccttcctgaggatcgtgcagtgcagaagcgtggagggcagctgcggcttcagctccagcagcaaggcccctcccccgagcctgccctccccaagcaggctgcctgggccctccgacacaccaatcctgcctcagtgatgaaggtctggatgcggccgc

SEQ ID NO: 16 - DNA, 937 bp, Homo sapiens
tctagaggacatggccaccggcagcaggaccagcctgctgctggccttcggcctgctgtgcctgccatggctgcaggagggcagcgccagctcttcttctaaggctccacccccatctctgcccagccccagcagactgccgggccccagcgacacacccattctgccccagttccccaccatccccctgagcaggctgttcgacaacgccatgctgagggctcacaggctgcaccagctggcctttgacacctaccaggagttcgaggaagcctacatccccaaggagcagaagtacagcttcctgcagaacccccagacctccctgtgcttcagcgagagcatccccacccccagcaacagagaggagacccagcagaagagcaacctggagctgctgaggatctccctgctgctgatccagagctggctggagcccgtgcagttcctgagaagcgtgttcgccaacagcctggtgtacggcgccagcgacagcaacgtgtacgacctgctgaaggacctggaggagggcatccagaccctgatgggccggctggaggacggcagccccaggaccggccagatcttcaagcagacctacagcaagttcgacaccaacagccacaacgacgacgccctgctgaagaactacgggctgctgtactgcttcagaaaggacatggacaaggtggagaccttcctgaggatcgtgcagtgcagaagcgtggagggcagctgcggcttcagctccagcagcaaggcccctcccccgagcctgccctccccaagcaggctgcctgggccctccgacacaccaatcctgccacagagcagctcctctaaggcccctcctccatccctgccatccccctcccggctgcctggcccctctgacacccctatcctgcctcagtgatgaaggtctggatgcggccgc

SEQ ID NO: 17 - DNA, 889 bp, Homo sapiens
tctagaggacatggccaccggcagcaggaccagcctgctgctggccttcggcctgctgtgcctgccatggctgcaggagggcagcgccagctcttcttctaaggctccacccccgagcctgcccttccccaccatccccctgagcaggctgttcgacaacgccatgctgagggctcacaggctgcaccagctggcctttgacacctaccaggagttcgaggaagcctacatccccaaggagcagaagtacagcttcctgcagaacccccagacctccctgtgcttcagcgagagcatccccacccccagcaacagagaggagacccagcagaagagcaacctggagctgctgaggatctccctgctgctgatccagagctggctggagcccgtgcagttcctgagaagcgtgttcgccaacagcctggtgtacggcgccagcgacagcaacgtgtacgacctgctgaaggacctggaggagggcatccagaccctgatgggccggctggaggacggcagccccaggaccggccagatcttcaagcagacctacagcaagttcgacaccaacagccacaacgacgacgccctgctgaagaactacgggctgctgtactgcttcagaaaggacatggacaaggtggagaccttcctgaggatcgtgcagtgcagaagcgtggagggcagctgcggcttcagctccagcagcaaggcccctcccccgagcctgccctccccaagcaggctgcctgggccctccgacacaccaatcctgccacagagcagctcctctaaggcccctcctccatccctgccatccccctcccggctgcctggcccctctgacacccctatcctgcctcagtgatgaaggtctggatgcggccgc

SEQ ID NO: 18 - DNA, 19 bp, Artificial Sequence
  XbaI Forward primer for HGH-CTP constructs
ctctagaggacatggccac

SEQ ID NO: 19 - DNA, 24 bp, Artificial Sequence
  Reverse primer for HGH-CTP constructs
acagggaggtctgggggttctgca

SEQ ID NO: 20 - DNA, 26 bp, Artificial Sequence
  Forward primer for HGH-CTP constructs
tgcagaacccccagacctccctgtgc

SEQ ID NO: 21 - DNA, 22 bp, Artificial Sequence
  Reverse primer for HGH-CTP constructs
ccaaactcatcaatgtatctta

SEQ ID NO: 22 - DNA, 19 bp, Artificial Sequence
  XbaI Forward primer for HGH-CTP constructs
ctctagaggacatggccac

SEQ ID NO: 23 - DNA, 25 bp, Artificial Sequence
  Reverse primer for HGH-CTP constructs
cgaactcctggtaggtgtcaaaggc

SEQ ID NO: 24 - DNA, 25 bp, Artificial Sequence
  Forward primer for HGH-CTP constructs
gcctttgacacctaccaggagttcg

SEQ ID NO: 25 - DNA, 33 bp, Artificial Sequence
  Reverse primer for HGH-CTP constructs
acgcggccgcatccagaccttcatcactgaggc

SEQ ID NO: 26 - DNA, 34 bp, Artificial Sequence
  Reverse primer for HGH-CTP constructs
gcggccgcggactcatcagaagccgcagctgccc